European Patent Application EP 4 643 870 A1, published November 5, 2025. Title: PEPTIDES AND USE THEREOF. Applicant: ステムリム株式会社. The sequence listing filed with the application follows.

SEQUENCE LISTING (28 sequences)

SEQ ID NO: 1 - protein, 30 aa, synthetic construct
FKDHKHIDVKDRHRTRHLAKTRCYHIDPHH

SEQ ID NO: 2 - DNA, 90 bp, synthetic construct
  source 1..90: mol_type = other DNA
tttaaagatcataaacatattgatgttaaagatcgtcatcgtactcgtcatcttgctaaaactcgttgttatcatattgatcctcatcat

SEQ ID NO: 3 - protein, 29 aa, synthetic construct
FKHKHIDVKDRHRTRHLAKTRCYHIDPHH

SEQ ID NO: 4 - DNA, 87 bp, synthetic construct
  source 1..87: mol_type = other DNA
tttaaacataaacatattgatgttaaagatcgtcatcgtactcgtcatcttgctaaaactcgttgttatcatattgatcctcatcat

SEQ ID NO: 5 - protein, 29 aa, synthetic construct
FKDHKHIVKDRHRTRHLAKTRCYHIDPHH

SEQ ID NO: 6 - DNA, 87 bp, synthetic construct
  source 1..87: mol_type = other DNA
tttaaagatcataaacatattgttaaagatcgtcatcgtactcgtcatcttgctaaaactcgttgttatcatattgatcctcatcat

SEQ ID NO: 7 - protein, 29 aa, synthetic construct
FKDHKHIDVKRHRTRHLAKTRCYHIDPHH

SEQ ID NO: 8 - DNA, 87 bp, synthetic construct
  source 1..87: mol_type = other DNA
tttaaagatcataaacatattgatgttaaacgtcatcgtactcgtcatcttgctaaaactcgttgttatcatattgatcctcatcat

SEQ ID NO: 9 - protein, 29 aa, synthetic construct
FKDHKHIDVKDRHRTRHLAKTRCYHIPHH

SEQ ID NO: 10 - DNA, 87 bp, synthetic construct
  source 1..87: mol_type = other DNA
tttaaagatcataaacatattgatgttaaagatcgtcatcgtactcgtcatcttgctaaaactcgttgttatcatattcctcatcat

SEQ ID NO: 11 - protein, 29 aa, synthetic construct
FKDKHIDVKDRHRTRHLAKTRCYHIDPHH

SEQ ID NO: 12 - DNA, 87 bp, synthetic construct
  source 1..87: mol_type = other DNA
tttaaagataaacatattgatgttaaagatcgtcatcgtactcgtcatcttgctaaaactcgttgttatcatattgatcctcatcat

SEQ ID NO: 13 - protein, 30 aa, synthetic construct
FKDHKHIDVKDRHRTRHLAKTRSYHIDPHH

SEQ ID NO: 14 - DNA, 90 bp, synthetic construct
  source 1..90: mol_type = other DNA
tttaaagatcataaacatattgatgttaaagatcgtcatcgtactcgtcatcttgctaaaactcgttcttatcatattgatcctcatcat

SEQ ID NO: 15 - protein, 30 aa, synthetic construct
FKDHKHIDVKDRHRTRHLAKTRAYHIDPHH

SEQ ID NO: 16 - DNA, 90 bp, synthetic construct
  source 1..90: mol_type = other DNA
tttaaagatcataaacatattgatgttaaagatcgtcatcgtactcgtcatcttgctaaaactcgtgcttatcatattgatcctcatcat

SEQ ID NO: 17 - protein, 30 aa, synthetic construct
FKDHKHIDVKDRHRTRHLAKTRTYHIDPHH

SEQ ID NO: 18 - DNA, 90 bp, synthetic construct
  source 1..90: mol_type = other DNA
tttaaagatcataaacatattgatgttaaagatcgtcatcgtactcgtcatcttgctaaaactcgtacttatcatattgatcctcatcat

SEQ ID NO: 19 - protein, 27 aa, synthetic construct
FKHKHIVKRHRTRHLAKTRCYHIDPHH

SEQ ID NO: 20 - DNA, 81 bp, synthetic construct
  source 1..81: mol_type = other DNA
tttaaacataaacatattgttaaacgtcatcgtactcgtcatcttgctaaaactcgttgttatcatattgatcctcatcat

SEQ ID NO: 21 - protein, 27 aa, synthetic construct
FKHKHIVKDRHRTRHLAKTRCYHIPHH

SEQ ID NO: 22 - DNA, 81 bp, synthetic construct
  source 1..81: mol_type = other DNA
tttaaacataaacatattgttaaagatcgtcatcgtactcgtcatcttgctaaaactcgttgttatcatattcctcatcat

SEQ ID NO: 23 - protein, 27 aa, synthetic construct
FKHKHIDVKRHRTRHLAKTRCYHIPHH

SEQ ID NO: 24 - DNA, 81 bp, synthetic construct
  source 1..81: mol_type = other DNA
tttaaacataaacatattgatgttaaacgtcatcgtactcgtcatcttgctaaaactcgttgttatcatattcctcatcat

SEQ ID NO: 25 - protein, 27 aa, synthetic construct
FKDHKHIVKRHRTRHLAKTRCYHIPHH

SEQ ID NO: 26 - DNA, 81 bp, synthetic construct
  source 1..81: mol_type = other DNA
tttaaagatcataaacatattgttaaacgtcatcgtactcgtcatcttgctaaaactcgttgttatcatattcctcatcat

SEQ ID NO: 27 - protein, 26 aa, synthetic construct
FKHKHIVKRHRTRHLAKTRCYHIPHH

SEQ ID NO: 28 - DNA, 78 bp, synthetic construct
  source 1..78: mol_type = other DNA
tttaaacataaacatattgttaaacgtcatcgtactcgtcatcttgctaaaactcgttgttatcatattcctcatcat